European Patent Specification EP 2 910 641 B1, published July 26, 2023. Title: HIGH MOLECULAR WEIGHT PHA-PRODUCING MICROBE AND METHOD OF PRODUCING HIGH MOLECULAR WEIGHT PHA USING SAME. Applicant: KANEKA CORPORATION. Application PCT/JP2013/078520. The sequence listing filed with the application follows.

SEQUENCE LISTING (19 sequences)

SEQ ID NO: 1 - DNA, 1089 bp, Cupriavidus necator
atgaccaaaagctttgccgctgactggcacgcgcagatccggcgactgagccgtgcgcaagcccgcacggaagcccaggtgaagtcctggctggaccgcgtggattcgcttaatccgctcacgccggctcggcctgaccgcccgccgggcaaggtccggcccgcccggccagcacccgcgccgggttccctgcccggtacctggcaggcgcacaggctgcgcctggcgccgctgccgggcgaactggtgccgcaactctcgtatcacctctacataccgtccaaggcccatcgcggcccgttgccggtggtggtggtgctgcatggctgtcgccagacgccggatgacctgtcggccggcacccgcatgaatgcgctggccgagcgcgagggatttatcgtggcctacccgcaacagcccttgcggcgccaggtgcagcgctgctggcagtggttcgacctgggcgccgctgagggcggacgcgaggcgcaggcggtggccgcgctgatcgatgcgctggctgcgcgccacgacgtgcgcgagcgcgagatctacctggccggcatgtccgccggcgcggccatggccgcggtggtggcgttgcgctacccgggcaaggtggcggccgcggcgctgcattccggcgtggtcatcggcgccgccgacaacccgcgcgccggcctgcgggccatgcagcaaggctcggcggccgatccgtcatggctgctggatgccgccggcgtgacgccgggcggtcccgagatgcccgcgctggtgatccacggcctggccgacgacgcggtccatccggtcaatggccgtctgctggcgcggcagttcctggcttacaacggcctggaagaccggctcgccggtgcgcccgcgcagtccggcccggaggacgaagcgccgggccggtctcatgaataccgcttcggccgctggcgccgcgacctggtcacgctggtggaagtggagggcttgggccacgcctggagcggcggcgatgccagctatggctaccacagcgatatcggcccggatgccagcacgatgatgtggcagttcttcagccagcaccgccgttga

SEQ ID NO: 2 - protein, 362 aa, Cupriavidus necator
MTKSFAADWHAQIRRLSRAQARTEAQVKSWLDRVDSLNPLTPARPDRPPGKVRPARPAPAPGSLPGTWQAHRLRLAPLPGELVPQLSYHLYIPSKAHRGPLPVVVVLHGCRQTPDDLSAGTRMNALAEREGFIVAYPQQPLRRQVQRCWQWFDLGAAEGGREAQAVAALIDALAARHDVREREIYLAGMSAGAAMAAVVALRYPGKVAAAALHSGVVIGAADNPRAGLRAMQQGSAADPSWLLDAAGVTPGGPEMPALVIHGLADDAVHPVNGRLLARQFLAYNGLEDRLAGAPAQSGPEDEAPGRSHEYRFGRWRRDLVTLVEVEGLGHAWSGGDASYGYHSDIGPDASTMMWQFFSQHRR

SEQ ID NO: 3 - DNA, 32 bp, Artificial
  primer1
gcgcatttaaatccggaccttcgtgcggctca

SEQ ID NO: 4 - DNA, 20 bp, Artificial
  primer2
gaggactcctgatcgtgtga

SEQ ID NO: 5 - DNA, 40 bp, Artificial
  primer3
tcacacgatcaggagtcctcagtcgggcagcaccaatgcg

SEQ ID NO: 6 - DNA, 32 bp, Artificial
  primer4
gcgcatttaaatcgccacgctgtgcctgacga

SEQ ID NO: 7 - DNA, 34 bp, Artificial
  primer5
gcgcgcatttaaatcatggcatctacgccgtcgg

SEQ ID NO: 8 - DNA, 20 bp, Artificial
  primer6
gccttttctgcctgggtcta

SEQ ID NO: 9 - DNA, 40 bp, Artificial
  primer7
tagacccaggcagaaaaggcgaaaacgcccgcgattgcgg

SEQ ID NO: 10 - DNA, 34 bp, Artificial
  primer8
gcgcgcatttaaatacgctggcgcgtttcgtctg

SEQ ID NO: 11 - DNA, 32 bp, Artificial
  primer9
aaatagatttaaatgggacagcagcaggattt

SEQ ID NO: 12 - DNA, 38 bp, Artificial
  primer10
gctggcggctgccgggggctcggtccccgctattctgg

SEQ ID NO: 13 - DNA, 38 bp, Artificial
  primer11
ccagaatagcggggaccgagcccccggcagccgccagc

SEQ ID NO: 14 - DNA, 33 bp, Artificial
  primer12
aaatagatttaaatacaaaggcaaaggggtagc

SEQ ID NO: 15 - protein, 594 aa, Aeromonas caviae
MSQPSYGPLFEALAHYNDKLLAMAKAQTERTAQALLQTNLDDLGQVLEQGSQQPWQLIQAQMNWWQDQLKLMQHTLLKSAGQPSEPVITPERSDRRFKAEAWSEQPIYDYLKQSYLLTARHLLASVDALEGVPQKSRERLRFFTRQYVSAMAPSNFLATNPELLKLTLESGGQNLVRGLALLAEDLERSADQLNIRLTDESAFELGRDLALTPGRVVQRTELYELIQYSPTTETVGKTPVLIVPPFINKYYIMDMRPQNSLVAWLVAQGQTVFMISWRNPGVAQAQIDLDDYVVDGVIAALDGVEAATGEREVHGIGYCIGGTALSLAMGWLAARRQKQRVRTATLFTTLLDFSQPGELGIFIHEPIIAALEAQNEAKGIMDGRQLAVSFSLLRENSLYWNYYIDSYLKGQSPVAFDLLHWNSDSTNVAGKTHNSLLRRLYLENQLVKGELKIRNTRIDLGKVKTPVLLVSAVDDHIALWQGTWQGMKLFGGEQRFLLAESGHIAGIINPPAANKYGFWHNGAEAESPESWLAGATHQGGSWWPEMMGFIQNRDEGSEPVPARVPEEGLAPAPGHYVKVRLNPVFACPTEEDAA

SEQ ID NO: 16 - DNA, 1260 bp, Cupriavidus necator
atgctctaccaattgcatgagttccagcgctcgatcctgcacccgctgaccgcgtgggcccaggcgaccgccaagaccttcaccaaccccctcagcccgctctcgctggttcccggcgcaccccgcctggctgccggctatgaactgctgtaccggctcggcaaggaatacgaaaagccggcattcgacatcaagtcggtgcgctccaacgggcgcgacatccccatcgtcgagcagaccgtgcttgaaaagccgttctgcaagctggtgcgcttcaagcgctatgccgacgacccggagaccatcaagctgctcaaggatgagccggtggtgctggtggccgcgccgctgtcgggccaccatgccacgctgctgcgcgacacggtgcgcacgctgctgcaggaccacaaggtctacgtcaccgactggatcgacgcacgcatggtgccggtcgaggaaggcgcgttccacctgtcggactacatctactacatccaggaattcatccgccatatcggcgccgagaacctgcatgtgatctcggtatgccagcccaccgtgccggtgctggccgcgatctcgctgatggcctcggccggcgagaagacgccgcgcaccatgaccatgatgggcggcccgatcgacgcccgcaagagccccaccgcggtcaactcgctggcgaccaacaagtcgttcgagtggttcgagaacaacgtcatctacaccgtgccggccaactaccccggccacggccgccgcgtctacccgggctttttgcagcatgccggtttcgtggcgatgaacccggaccggcacctttcctcgcactatgacttctacctgagcctggtcgagggcgatgcggatgacgccgaagcccacgtgcgcttctacgacgaatacaacgcggtgctcgacatggccgccgagtactacctcgacaccatccgcgaggtgttccaggaattccgcctggccaacggcacctgggccatcgacggcaatccggtgcggccgcaggacatcaagagcaccgcgctgatgaccgtcgagggcgaactggacgacatctcgggcgcgggccagaccgccgcggcgcacgacctgtgcgccggcatcccgaaaatccgcaagcagcacctgaacgcggcacactgcggccactacggcatcttctcgggccggcgctggcgcgaagagatctacccgcagctgcgcgactttatccgcaagtaccaccaggcctcggccaccaggtaa

SEQ ID NO: 17 - protein, 419 aa, Cupriavidus necator
MLYQLHEFQRSILHPLTAWAQATAKTFTNPLSPLSLVPGAPRLAAGYELLYRLGKEYEKPAFDIKSVRSNGRDIPIVEQTVLEKPFCKLVRFKRYADDPETIKLLKDEPVVLVAAPLSGHHATLLRDTVRTLLQDHKVYVTDWIDARMVPVEEGAFHLSDYIYYIQEFIRHIGAENLHVISVCQPTVPVLAAISLMASAGEKTPRTMTMMGGPIDARKSPTAVNSLATNKSFEWFENNVIYTVPANYPGHGRRVYPGFLQHAGFVAMNPDRHLSSHYDFYLSLVEGDADDAEAHVRFYDEYNAVLDMAAEYYLDTIREVFQEFRLANGTWAIDGNPVRPQDIKSTALMTVEGELDDISGAGQTAAAHDLCAGIPKIRKQHLNAAHCGHYGIFSGRRWREEIYPQLRDFIRKYHQASATR

SEQ ID NO: 18 - DNA, 1260 bp, Cupriavidus necator
atgcatattgcggctcgcaagaaccagaatagcggggaccgagccatgctgtaccacgcctaccagatctacgcggacatgatactgccggcctgcacgctggcggagctggctgccgcgacgctggcggcaaatcccaggtccggtggtttcgacgcggtgccccgcctgcgtgccgcctgcgagctcatcgcactggtgcggctcacgcaccaccggccggccttcggcatcgaccacgcaaccgtcggcggccagccggtgccggtcaccgaggaagtcgtcgcgcgcacgccgttctgctcgctgctgcacttccgccgccacggcatcgtcggccagccgcgcgtgctgctggtggcgccgatgtccggccacttcgccacgctgctgcgcggcacggtccagaccatgctggccgaccacgacgtctatctcaccgactggcacaacccccgcgacattccgttgctggccgggcgcttcggcttcgatgaattcgtgcagcacctgatcggcttcctgcagacgctgggcggaggcacgcatctggtggcgatttgccagcctgccgtggcagcgctggcggcagcggcactcatggccgaggacggggatcccgcccagccgcccagcctgacgctgatggccggccccatcgacgcgcgcgtcaatccgaccaaggtcaacgcgctggccatgagccaacccctcgaatggttcgagcgcaccttgatcggcatggtgccgctgcgctttgccggcgcgatgcggcgcgtctacccgggccacgtgcagctgctggccttcatgagcatgaacccggagcggcacgaacaggcgctgcgcgagctctacgccctgcgcgagcgcggcgagcacgacaaggccgatgccatccgcgacttctacatcgagtacttcgccaccatggacctgaccgcggagttctacctggaaaccgtcagcctggtattccagcgcttcctgctggcccagggcctgcttgacgtgagcggacgccgtgtccgcacgcgcgccatccaccgcaccgccctgctcaccgtggagggtgaacgcgacgatatctgcgccatcggccagaccgtggcggcgcaggacctgtgctccagcctgcgcccctacatgcgcatgcatcatgtgcagaccggggtcgggcactatggcgtgttcaacggcaggcggtgggagacgcaggtgtacccgctggtgcgcaacaccatctacaccagcagctaa

SEQ ID NO: 19 - protein, 419 aa, Cupriavidus necator
MHIAARKNQNSGDRAMLYHAYQIYADMILPACTLAELAAATLAANPRSGGFDAVPRLRAACELIALVRLTHHRPAFGIDHATVGGQPVPVTEEVVARTPFCSLLHFRRHGIVGQPRVLLVAPMSGHFATLLRGTVQTMLADHDVYLTDWHNPRDIPLLAGRFGFDEFVQHLIGFLQTLGGGTHLVAICQPAVAALAAAALMAEDGDPAQPPSLTLMAGPIDARVNPTKVNALAMSQPLEWFERTLIGMVPLRFAGAMRRVYPGHVQLLAFMSMNPERHEQALRELYALRERGEHDKADAIRDFYIEYFATMDLTAEFYLETVSLVFQRFLLAQGLLDVSGRRVRTRAIHRTALLTVEGERDDICAIGQTVAAQDLCSSLRPYMRMHHVQTGVGHYGVFNGRRWETQVYPLVRNTIYTSS